European Patent Application EP 4 644 418 A1, published November 5, 2025. Title: 靶向BCMA的纳米抗体、嵌合抗原受体及其应用. Applicant: 河北森朗生物科技有限公司. The sequence listing filed with the application follows.

SEQUENCE LISTING (33 sequences)

SEQ ID NO: 1 - protein, 121 aa, Artificial sequence
QVQLQESGGGSVQPGGSLRLSCKASGFTFSPSAMSWARQAPGKEIEWVSNIYPDGRTYYADSMKGRFTISRDNAENTVYLQMNSLKPEDTAVYYCLIGVGIVAGQVVSPYWGQGTQVTVSS

SEQ ID NO: 2 - DNA, 363 bp, Artificial sequence
  source 1..363: mol_type = other DNA
caggtgcagctgcaggagtctggaggaggctcggtacagcctggggggtctctgagactctcctgtaaagcctctggattcaccttcagtccctctgccatgagctgggcccgccaggcaccagggaaggagatcgagtgggtgtccaatatttaccctgatggacgcacatactatgcggactccatgaagggccgattcaccatctccagagacaacgccgagaacacggtgtatctgcaaatgaacagcctgaaacctgaggacacggccgtttattactgtctaataggagtcggtattgtggccggtcaggtagtttcgccctactggggtcaggggacccaggtcaccgtctcctca

SEQ ID NO: 3 - protein, 8 aa, Artificial sequence
GFTFSPSA

SEQ ID NO: 4 - DNA, 24 bp, Artificial sequence
  source 1..24: mol_type = other DNA
ggattcaccttcagtccctctgcc

SEQ ID NO: 5 - protein, 7 aa, Artificial sequence
IYPDGRT

SEQ ID NO: 6 - DNA, 21 bp, Artificial sequence
  source 1..21: mol_type = other DNA
atttaccctgatggacgcaca

SEQ ID NO: 7 - protein, 15 aa, Artificial sequence
LIGVGIVAGQVVSPY

SEQ ID NO: 8 - DNA, 45 bp, Artificial sequence
  source 1..45: mol_type = other DNA
ctaataggagtcggtattgtggccggtcaggtagtttcgccctac

SEQ ID NO: 9 - protein, 124 aa, Artificial sequence
QVQLQESGGGLVQPGGSLRLSCAASGFTFSNYAMSWFRQGPGKERELVAGIDRTGGSTRTADSVQGRFTISRDNAKNKVYLQMNSLKPEDTAVYYCKALRTPGWGTSPDVVGYWGQGTQVTVSS

SEQ ID NO: 10 - DNA, 372 bp, Artificial sequence
  source 1..372: mol_type = other DNA
caggtgcagctgcaggagtctggaggaggcttggtgcagcctggggggtctctgagactctcctgtgcagcctctggattcaccttcagtaactatgccatgagctggttccgccagggtccagggaaggagcgcgagttggtcgcaggtatcgatcgtactggaggtagcacaaggactgcagactccgtgcagggccgattcaccatctccagagacaatgccaagaacaaggtgtatctgcaaatgaatagcctgaaacctgaggacacggccgtgtattattgtaaggcactgaggactccgggctggggtacgtctcccgatgtcgttggctactggggccaggggacccaggtcaccgtctcctca

SEQ ID NO: 11 - protein, 8 aa, Artificial sequence
GFTFSNYA

SEQ ID NO: 12 - DNA, 24 bp, Artificial sequence
  source 1..24: mol_type = other DNA
ggattcaccttcagtaactatgcc

SEQ ID NO: 13 - protein, 8 aa, Artificial sequence
IDRTGGST

SEQ ID NO: 14 - DNA, 24 bp, Artificial sequence
  source 1..24: mol_type = other DNA
atcgatcgtactggaggtagcaca

SEQ ID NO: 15 - protein, 17 aa, Artificial sequence
KALRTPGWGTSPDVVGY

SEQ ID NO: 16 - DNA, 51 bp, Artificial sequence
  source 1..51: mol_type = other DNA
aaggcactgaggactccgggctggggtacgtctcccgatgtcgttggctac

SEQ ID NO: 17 - DNA, 1179 bp, Artificial sequence
  source 1..1179: mol_type = other DNA
ggctccggtgcccgtcagtgggcagagcgcacatcgcccacagtccccgagaagttggggggaggggtcggcaattgaaccggtgcctagagaaggtggcgcggggtaaactgggaaagtgatgtcgtgtactggctccgcctttttcccgagggtgggggagaaccgtatataagtgcagtagtcgccgtgaacgttctttttcgcaacgggtttgccgccagaacacaggtaagtgccgtgtgtggttcccgcgggcctggcctctttacgggttatggcccttgcgtgccttgaattacttccacctggctgcagtacgtgattcttgatcccgagcttcgggttggaagtgggtgggagagttcgaggccttgcgcttaaggagccccttcgcctcgtgcttgagttgaggcctggcctgggcgctggggccgccgcgtgcgaatctggtggcaccttcgcgcctgtctcgctgctttcgataagtctctagccatttaaaatttttgatgacctgctgcgacgctttttttctggcaagatagtcttgtaaatgcgggccaagatctgcacactggtatttcggtttttggggccgcgggcggcgacggggcccgtgcgtcccagcgcacatgttcggcgaggcggggcctgcgagcgcggccaccgagaatcggacgggggtagtctcaagctggccggcctgctctggtgcctggcctcgcgccgccgtgtatcgccccgccctgggcggcaaggctggcccggtcggcaccagttgcgtgagcggaaagatggccgcttcccggccctgctgcagggagctcaaaatggaggacgcggcgctcgggagagcgggcgggtgagtcacccacacaaaggaaaagggcctttccgtcctcagccgtcgcttcatgtgactccacggagtaccgggcgccgtccaggcacctcgattagttctcgagcttttggagtacgtcgtctttaggttggggggaggggttttatgcgatggagtttccccacactgagtgggtggagactgaagttaggccagcttggcacttgatgtaattctccttggaatttgccctttttgagtttggatcttggttcattctcaagcctcagacagtggttcaaagtttttttcttccatttcaggtgtcgtga

SEQ ID NO: 18 - protein, 22 aa, Artificial sequence
MLLLVTSLLLCELPHPAFLLIP

SEQ ID NO: 19 - protein, 46 aa, Artificial sequence
TTPAPRPPTPAPTIASQPLSLRPEACRPAAGGAVHTRGLDFACDIY

SEQ ID NO: 20 - protein, 24 aa, Artificial sequence
IWAPLAGTCGVLLLSLVITLYCKR

SEQ ID NO: 21 - protein, 42 aa, Artificial sequence
GRKKLLYIFKQPFMRPVQTTQEEDGCSCRFPEEEEGGCELRV

SEQ ID NO: 22 - protein, 110 aa, Artificial sequence
KFSRSADAPAYKQGQNQLYNELNLGRREEYDVLDKRRGRDPEMGGKPRRKNPQEGLYNELQKDKMAEAYSEIGMKGERRRGKGHDGLYQGLSTATKDTYDALHMQALPPR

SEQ ID NO: 23 - protein, 23 aa, Artificial sequence
LEGGGEGRGSLLTCGDVEENPGP

SEQ ID NO: 24 - protein, 23 aa, Artificial sequence
RMLLLVTSLLLCELPHPAFLLIP

SEQ ID NO: 25 - protein, 335 aa, Artificial sequence
RKVCNGIGIGEFKDSLSINATNIKHFKNCTSISGDLHILPVAFRGDSFTHTPPLDPQELDILKTVKEITGFLLIQAWPENRTDLHAFENLEIIRGRTKQHGQFSLAVVSLNITSLGLRSLKEISDGDVIISGNKNLCYANTINWKKLFGTSGQKTKIISNRGENSCKATGQVCHALCSPEGCWGPEPRDCVSCRNVSRGRECVDKCNLLEGEPREFVENSECIQCHPECLPQAMNITCTGRGPDNCIQCAHYIDGPHCVKTCPAGVMGENNTLVWKYADAGHVCHLCHPNCTYGCTGPGLEGCPTNGPKIPSIATGMVGALLLLLVVALGIGLFM

SEQ ID NO: 26 - DNA, 66 bp, Artificial sequence
  source 1..66: mol_type = other DNA
atgctgctgctggtgaccagcctgctgctgtgcgagctgccccaccccgcctttctgctgatcccc

SEQ ID NO: 27 - DNA, 138 bp, Artificial sequence
  source 1..138: mol_type = other DNA
actaccccagcaccgcggccgcccaccccggctcctaccatcgcctcccagcctctgtccctgcgtccggaggcatgtagacccgcagctggtggggccgtgcatacccggggtcttgacttcgcctgcgatatctac

SEQ ID NO: 28 - DNA, 72 bp, Artificial sequence
  source 1..72: mol_type = other DNA
atttgggcccctctggctggtacttgcggggtcctgctgctttcactcgtgatcactctttactgtaagcgc

SEQ ID NO: 29 - DNA, 126 bp, Artificial sequence
  source 1..126: mol_type = other DNA
ggtcggaagaagctgctgtacatctttaagcaacccttcatgaggcctgtgcagactactcaagaggaggacggctgttcatgccggttcccagaggaggaggaaggcggctgcgaactgcgcgtg

SEQ ID NO: 30 - DNA, 330 bp, Artificial sequence
  source 1..330: mol_type = other DNA
aaattcagccgcagcgcagatgctccagcctacaagcaggggcagaaccagctctacaacgaactcaatcttggtcggagagaggagtacgacgtgctggacaagcggagaggacgggacccagaaatgggcgggaagccgcgcagaaagaatccccaagagggcctgtacaacgagctccaaaaggataagatggcagaagcctatagcgagattggtatgaaaggggaacgcagaagaggcaaaggccacgacggactgtaccagggactcagcaccgccaccaaggacacctatgacgctcttcacatgcaggccctgccgcctcgg

SEQ ID NO: 31 - DNA, 69 bp, Artificial sequence
  source 1..69: mol_type = other DNA
ctcgagggcggcggagagggcagaggaagtcttctaacatgcggtgacgtggaggagaatcccggccct

SEQ ID NO: 32 - DNA, 69 bp, Artificial sequence
  source 1..69: mol_type = other DNA
aggatgcttctcctggtgacaagccttctgctctgtgagttaccacacccagcattcctcctgatccca

SEQ ID NO: 33 - DNA, 1005 bp, Artificial sequence
  source 1..1005: mol_type = other DNA
cgcaaagtgtgtaacggaataggtattggtgaatttaaagactcactctccataaatgctacgaatattaaacacttcaaaaactgcacctccatcagtggcgatctccacatcctgccggtggcatttaggggtgactccttcacacatactcctcctctggatccacaggaactggatattctgaaaaccgtaaaggaaatcacagggtttttgctgattcaggcttggcctgaaaacaggacggacctccatgcctttgagaacctagaaatcatacgcggcaggaccaagcaacatggtcagttttctcttgcagtcgtcagcctgaacataacatccttgggattacgctccctcaaggagataagtgatggagatgtgataatttccggaaacaaaaatttgtgctatgcaaatacaataaactggaaaaaactgtttgggacctccggtcagaaaaccaaaattataagcaacagaggtgaaaacagctgcaaggccacaggccaggtctgccatgccttgtgctcccccgagggctgctggggcccggagcccagggactgcgtctcttgccggaatgtcagccgaggcagggaatgcgtggacaagtgcaaccttctggagggtgagccaagggagtttgtggagaactctgagtgcatacagtgccacccagagtgcctgcctcaggccatgaacatcacctgcacaggacggggaccagacaactgtatccagtgtgcccactacattgacggcccccactgcgtcaagacctgcccggcaggagtcatgggagaaaacaacaccctggtctggaagtacgcagacgccggccatgtgtgccacctgtgccatccaaactgcacctacggatgcactgggccaggtcttgaaggctgtccaacgaatgggcctaagatcccgtccatcgccactgggatggtgggggccctcctcttgctgctggtggtggccctggggatcggcctcttcatg